European Patent Application EP 4 803 094 A2, published September 9, 2026. Title: NOVEL GLP-1/GIP DUAL, GLP-1/GCG DUAL AND GLP-1/GIP/GCG TRIPLE RECEPTOR AGONISTS. Applicant: Sun Pharmaceutical Industries Ltd. Application IB. The sequence listing filed with the application follows.

SEQUENCE LISTING (32 sequences)

SEQ ID NO: 1 - protein, 39 aa, synthetic construct
  VARIANT 1: note = Y
  VARIANT 2: note = Aib
  VARIANT 3: note = Q; note = N
  VARIANT 10: note = Y
  VARIANT 12: note = I
  VARIANT 16: note = K
  VARIANT 17: note = I; note = K
  VARIANT 18: note = A
  VARIANT 19: note = Q
  VARIANT 21: note = A
  VARIANT 23: note = I; note = V
  VARIANT 24: note = Q; note = E
  VARIANT 25: note = Y; note = W
  VARIANT 27: note = I; note = L
  VARIANT 28: note = A; note = E
  VARIANT 29: note = G
  VARIANT 30: note = G
  VARIANT 31: note = P
  VARIANT 32: note = S
  VARIANT 33: note = S
  VARIANT 34: note = G
  VARIANT 35: note = A
  VARIANT 36: note = P
  VARIANT 37: note = P
  VARIANT 38: note = P
  VARIANT 39: note = S
  SITE 17: note = K is conjugated to a C16-C22 fatty acid.
  SITE 20: note = K is conjugated to a C16-C22 fatty acid.
  VARIANT 13: note = L-alpha-methylleucine; note = Nva
  VARIANT 20: note = L-alpha-methylleucine; note = Nva
XXXGTFTSDXSXXLDXXXXXXFXXXLXXXXXXXXXXXXX

SEQ ID NO: 2 - protein, 39 aa, synthetic construct; identical to SEQ ID NO: 1
  VARIANT 1: note = Y
  VARIANT 2: note = Aib
  VARIANT 3: note = Q; note = N
  VARIANT 10: note = Y
  VARIANT 12: note = I
  VARIANT 13: note = 2-amino-2,4-dimethylpentanoic acid
  VARIANT 16: note = K
  VARIANT 17: note = I; note = K
  VARIANT 18: note = A
  VARIANT 19: note = Q
  VARIANT 20: note = L; note = K
  VARIANT 21: note = A
  VARIANT 23: note = V; note = I
  VARIANT 24: note = E; note = Q
  VARIANT 25: note = Y; note = W
  VARIANT 27: note = L; note = I
  VARIANT 28: note = A; note = E
  VARIANT 29: note = G
  VARIANT 30: note = G
  VARIANT 31: note = P
  VARIANT 32: note = S
  VARIANT 33: note = S
  VARIANT 34: note = G
  VARIANT 35: note = A
  VARIANT 36: note = P
  VARIANT 37: note = P
  VARIANT 38: note = P
  VARIANT 39: note = S
  VARIANT 20: note = or L-alpha-methylleucine; note = Nva

SEQ ID NO: 3 - protein, 39 aa, synthetic construct; identical to SEQ ID NO: 1
  VARIANT 1: note = Y
  VARIANT 2: note = Aib
  VARIANT 3: note = N; note = Q
  VARIANT 10: note = Y
  VARIANT 12: note = I
  VARIANT 13: note = 2-amino-2,4-dimethylpentanoic acid; note = Serine methyl ester; note = Nle; note = Nva; note = Aib
  VARIANT 16: note = K
  VARIANT 17: note = I; note = K
  VARIANT 18: note = A
  VARIANT 19: note = Q
  VARIANT 20: note = Serine methyl ether; note = Nle; note = Nva; note = Aib; note = K
  VARIANT 21: note = A
  VARIANT 23: note = V; note = I
  VARIANT 24: note = Q; note = E
  VARIANT 25: note = W; note = Y
  VARIANT 27: note = E; note = L; note = I
  VARIANT 28: note = E; note = A
  VARIANT 29: note = G
  VARIANT 30: note = G
  VARIANT 31: note = P
  VARIANT 32: note = S
  VARIANT 33: note = S
  VARIANT 34: note = G
  VARIANT 35: note = A
  VARIANT 36: note = P
  VARIANT 37: note = P
  VARIANT 38: note = P
  VARIANT 39: note = S
  VARIANT 17: note = K is acylated with Moiety D; note = K is acylated with Moiety H; note = K is acylated with Moiety E; note = K is acylated with Moiety F; note = K is acylated with Moiety A; note = K is acylated with Moiety B; note = K is acylated with Moiety I; note = K is acylated with Moiety C; note = K is acylated with Moiety G
  VARIANT 20: note = K is acylated with Moiety F; note = K is acylated with Moiety G; note = K is acylated with Moiety H; note = K is acylated with Moiety I; note = K is acylated with Moiety A; note = K is acylated with Moiety C; note = K is acylated with Moiety D; note = K is acylated with Moiety B; note = K is acylated with Moiety E

SEQ ID NO: 4 - protein, 39 aa, synthetic construct; identical to SEQ ID NO: 1
  VARIANT 1: note = Y
  VARIANT 2: note = Aib
  VARIANT 3: note = Q; note = N
  VARIANT 10: note = Y
  VARIANT 12: note = I
  VARIANT 13: note = 2-amino-2,4-dimethylpentanoic acid; note = Nle; note = Nva
  VARIANT 16: note = K
  VARIANT 17: note = K; note = I
  VARIANT 18: note = A
  VARIANT 19: note = Q
  VARIANT 20: note = K; note = Aib
  VARIANT 21: note = A
  VARIANT 23: note = I; note = V
  VARIANT 24: note = E; note = Q
  VARIANT 25: note = Y; note = W
  VARIANT 27: note = I; note = L
  VARIANT 28: note = E; note = A
  VARIANT 29: note = G
  VARIANT 30: note = G
  VARIANT 31: note = P
  VARIANT 32: note = S
  VARIANT 33: note = S
  VARIANT 34: note = G
  VARIANT 35: note = A
  VARIANT 36: note = P
  VARIANT 37: note = P
  VARIANT 38: note = P
  VARIANT 39: note = S
  VARIANT 17: note = K is acylated with Moiety C; note = K is acylated with Moiety A; note = K is acylated with Moiety B; note = K is acylated with Moiety D

SEQ ID NO: 5 - protein, 39 aa, synthetic construct
  VARIANT 3: note = Q; note = N
  SITE 2: note = Aib
  VARIANT 13: note = Nva; note = 2-amino-2,4-dimethylpentanoic acid; note = Nle
  VARIANT 17: note = K; note = I
  VARIANT 20: note = Aib; note = K
  VARIANT 23: note = I; note = V
  VARIANT 24: note = E; note = Q
  VARIANT 25: note = W; note = Y
  VARIANT 27: note = I; note = L
  VARIANT 28: note = E; note = A
  VARIANT 17: note = K is acylated with Moiety B; note = K is acylated with Moiety H; note = K is acylated with Moiety A; note = K is acylated with Moiety D; note = K is acylated with Moiety C; note = K is acylated with Moiety G; note = K is acylated with Moiety I
  VARIANT 20: note = K is acylated with Moiety H; note = K is acylated with Moiety D; note = K is acylated with Moiety G; note = K is acylated with Moiety B; note = K is acylated with Moiety C; note = K is acylated with Moiety A; note = K is acylated with Moiety I
YXXGTFTSDYSIXLDKXAQXAFXXXLXXGGPSSGAPPPS

SEQ ID NO: 6 - protein, 39 aa, synthetic construct
  VARIANT 2: note = Aib
  VARIANT 3: note = N; note = Q
  VARIANT 13: note = 2-amino-2,4-dimethylpentanoic acid; note = Nva; note = Nle
  VARIANT 17: note = K
  VARIANT 20: note = Nva; note = Aib; note = Nle
  VARIANT 17: note = K is acylated with Moiety A; note = K is acylated with Moiety I; note = K is acylated with Moiety H
YXXGTFTSDYSIXLDKXAQXAFIEYLLEGGPSSGAPPPS

SEQ ID NO: 7 - protein, 38 aa, synthetic construct
  SITE 2: note = Aib
  SITE 13: note = 2-amino-2,4-dimethylpentanoic acid
  SITE 20: note = Aib
YXQGTFTSDYSIXLDKKAQXAFIEYLLEGGPSSGAPPP

SEQ ID NO: 8 - protein, 39 aa, synthetic construct
  SITE 2: note = Aib
  SITE 13: note = 2-amino-2,4-dimethylpentanoic acid
  SITE 20: note = Aib
  VARIANT 17: note = K is acylated with Moiety A; note = K is acylated with Moiety F; note = K is acylated with Moiety G; note = K is acylated with Moiety H; note = K is acylated with Moiety E; note = K is acylated with Moiety I; note = K is acylated with Moiety C; note = K is acylated with Moiety D; note = K is acylated with Moiety B
YXQGTFTSDYSIXLDKKAQXAFIEYLLEGGPSSGAPPPS

SEQ ID NO: 9 - protein, 39 aa, synthetic construct; identical to SEQ ID NO: 8
  SITE 2: note = Aib
  SITE 13: note = Nva
  SITE 20: note = Aib
  VARIANT 17: note = K is acylated with Moiety E; note = K is acylated with Moiety D; note = K is acylated with Moiety F; note = K is acylated with Moiety H; note = K is acylated with Moiety A; note = K is acylated with Moiety B; note = K is acylated with Moiety C; note = K is acylated with Moiety I; note = K is acylated with Moiety G

SEQ ID NO: 10 - protein, 39 aa, synthetic construct
  SITE 2: note = Aib
  SITE 13: note = Nva
  SITE 20: note = Aib
  VARIANT 17: note = K is acylated with Moiety E; note = K is acylated with Moiety D; note = K is acylated with Moiety A; note = K is acylated with Moiety I; note = K is acylated with Moiety G; note = K is acylated with Moiety C; note = K is acylated with Moiety B; note = K is acylated with Moiety H; note = K is acylated with Moiety F
YXNGTFTSDYSIXLDKKAQXAFIEYLLEGGPSSGAPPPS

SEQ ID NO: 11 - protein, 39 aa, synthetic construct; identical to SEQ ID NO: 8
  SITE 2: note = Aib
  SITE 13: note = Nle
  SITE 20: note = Aib
  VARIANT 17: note = K is acylated with Moiety E; note = K is acylated with Moiety I; note = K is acylated with Moiety G; note = K is acylated with Moiety B; note = K is acylated with Moiety F; note = K is acylated with Moiety H; note = K is acylated with Moiety A; note = K is acylated with Moiety C; note = K is acylated with Moiety D

SEQ ID NO: 12 - protein, 39 aa, synthetic construct; identical to SEQ ID NO: 8
  SITE 2: note = Aib
  SITE 13: note = 2-amino-2,4-dimethylpentanoic acid
  SITE 20: note = Nva
  VARIANT 17: note = K is acylated with Moiety H; note = K is acylated with Moiety G; note = K is acylated with Moiety A; note = K is acylated with Moiety I; note = K is acylated with Moiety F; note = K is acylated with Moiety B; note = K is acylated with Moiety D; note = K is acylated with Moiety C; note = K is acylated with Moiety E

SEQ ID NO: 13 - protein, 39 aa, synthetic construct; identical to SEQ ID NO: 10
  SITE 2: note = Aib
  SITE 13: note = 2-amino-2,4-dimethylpentanoic acid
  SITE 20: note = Nva
  VARIANT 17: note = K is acylated with Moiety C; note = K is acylated with Moiety A; note = K is acylated with Moiety D; note = K is acylated with Moiety F; note = K is acylated with Moiety G; note = K is acylated with Moiety I; note = K is acylated with Moiety H; note = K is acylated with Moiety B; note = K is acylated with Moiety E

SEQ ID NO: 14 - protein, 39 aa, synthetic construct; identical to SEQ ID NO: 8
  SITE 2: note = Aib
  SITE 13: note = Nva
  SITE 20: note = Nle
  VARIANT 17: note = K is acylated with Moiety H; note = K is acylated with Moiety E; note = K is acylated with Moiety B; note = K is acylated with Moiety C; note = K is acylated with Moiety D; note = K is acylated with Moiety A; note = K is acylated with Moiety F; note = K is acylated with Moiety G

SEQ ID NO: 15 - protein, 39 aa, synthetic construct
  SITE 2: note = Aib
  SITE 13: note = Nva
  VARIANT 17: note = K is acylated with Moiety H; note = K is acylated with Moiety D; note = K is acylated with Moiety B; note = K is acylated with Moiety A; note = K is acylated with Moiety F; note = K is acylated with Moiety I; note = K is acylated with Moiety E; note = K is acylated with Moiety C; note = K is acylated with Moiety G
YXQGTFTSDYSIXLDKIAQKAFVQWLIAGGPSSGAPPPS

SEQ ID NO: 16 - protein, 39 aa, synthetic construct; identical to SEQ ID NO: 15
  SITE 2: note = Aib
  SITE 13: note = Nva
  VARIANT 17: note = K is acylated with Moiety F; note = K is acylated with Moiety D; note = K is acylated with Moiety E; note = K is acylated with Moiety G; note = K is acylated with Moiety A; note = K is acylated with Moiety I; note = K is acylated with Moiety C; note = K is acylated with Moiety H; note = K is acylated with Moiety B

SEQ ID NO: 17 - protein, 39 aa, synthetic construct
  SITE 2: note = Aib
  SITE 13: note = 2-amino-2,4-dimethylpentanoic acid
  SITE 17: note = Moiety A
  SITE 20: note = Aib
YXQGTFTSDYSIXLDKXAQXAFIEYLLEGGPSSGAPPPS

SEQ ID NO: 18 - protein, 39 aa, synthetic construct; identical to SEQ ID NO: 17
  SITE 2: note = Aib
  SITE 13: note = 2-amino-2,4-dimethylpentanoic acid
  SITE 17: note = Moiety B
  SITE 20: note = Aib

SEQ ID NO: 19 - protein, 39 aa, synthetic construct; identical to SEQ ID NO: 17
  SITE 2: note = Aib
  SITE 13: note = 2-amino-2,4-dimethylpentanoic acid
  SITE 17: note = Moiety B
  SITE 20: note = Aib

SEQ ID NO: 20 - protein, 39 aa, synthetic construct; identical to SEQ ID NO: 17
  SITE 2: note = Aib
  SITE 13: note = Nle
  SITE 17: note = Moiety A
  SITE 20: note = Aib

SEQ ID NO: 21 - protein, 39 aa, synthetic construct; identical to SEQ ID NO: 17
  SITE 2: note = Aib
  SITE 13: note = Nva
  SITE 17: note = Moiety A
  SITE 20: note = Aib

SEQ ID NO: 22 - protein, 39 aa, synthetic construct; identical to SEQ ID NO: 17
  SITE 2: note = Aib
  SITE 13: note = Nva
  SITE 17: note = Moiety B
  SITE 20: note = Aib

SEQ ID NO: 23 - protein, 39 aa, synthetic construct; identical to SEQ ID NO: 17
  SITE 2: note = Aib
  SITE 13: note = Nva
  SITE 17: note = Moiety G
  SITE 20: note = Aib

SEQ ID NO: 24 - protein, 39 aa, synthetic construct; identical to SEQ ID NO: 17
  SITE 2: note = Aib
  SITE 13: note = 2-amino-2,4-dimethylpentanoic acid
  SITE 17: note = Moiety C
  SITE 20: note = Aib

SEQ ID NO: 25 - protein, 39 aa, synthetic construct; identical to SEQ ID NO: 17
  SITE 2: note = Aib
  SITE 13: note = 2-amino-2,4-dimethylpentanoic acid
  SITE 17: note = Moiety D
  SITE 20: note = Aib

SEQ ID NO: 26 - protein, 39 aa, synthetic construct
  SITE 2: note = Aib
  SITE 13: note = Nva
  SITE 20: note = Moiety A
YXQGTFTSDYSIXLDKIAQXAFVQWLIAGGPSSGAPPPS

SEQ ID NO: 27 - protein, 39 aa, synthetic construct; identical to SEQ ID NO: 26
  SITE 2: note = Aib
  SITE 13: note = Nva
  SITE 20: note = Moiety B

SEQ ID NO: 28 - protein, 39 aa, synthetic construct; identical to SEQ ID NO: 26
  SITE 2: note = Aib
  SITE 13: note = Nva
  SITE 20: note = Moiety B

SEQ ID NO: 29 - protein, 39 aa, synthetic construct; identical to SEQ ID NO: 26
  SITE 2: note = Aib
  SITE 13: note = Nva
  SITE 20: note = Moiety A

SEQ ID NO: 30 - protein, 39 aa, synthetic construct; identical to SEQ ID NO: 17
  SITE 2: note = Aib
  SITE 13: note = 2-amino-2,4-dimethylpentanoic acid
  SITE 17: note = Moiety G
  SITE 20: note = Aib

SEQ ID NO: 31 - protein, 6 aa, synthetic construct
GTFTSD

SEQ ID NO: 32 - protein, 11 aa, synthetic construct
GGPSSGAPPPS